European Patent Application EP 4 130 747 A1, published February 8, 2023. Title: Biomarkers for Cancer immunotherapy and Use thereof. Applicant: RopheLBio Co., Ltd. The sequence listing filed with the application follows.

SEQUENCE LISTING (26 sequences)

SEQ ID NO: 1 - DNA, 20 bp, Artificial Sequence
  Forward primer for mouse DRG2
tggaaccatccaaatccgcc

SEQ ID NO: 2 - DNA, 22 bp, Artificial Sequence
  Reverse primer for mouse DRG2
caagaaggtggacttacccaca

SEQ ID NO: 3 - DNA, 20 bp, Artificial Sequence
  Forward primer for mouse PD-L1
agcctggaacaacggacatt

SEQ ID NO: 4 - DNA, 20 bp, Artificial Sequence
  Reverse primer for mouse PD-L1
ctgctaagccaggaaccctc

SEQ ID NO: 5 - DNA, 20 bp, Artificial Sequence
  Forward primer for mouse PD-L2
ttattcaccgtgacagcccc

SEQ ID NO: 6 - DNA, 20 bp, Artificial Sequence
  Reverse primer for mouse PD-L2
agtgcattctctgcggtcaa

SEQ ID NO: 7 - DNA, 20 bp, Artificial Sequence
  Forward primer for mouse Gal9
gtgcagttctctcagccagt

SEQ ID NO: 8 - DNA, 20 bp, Artificial Sequence
  Reverse primer for mouse Gal9
gtgggcaggacgaaagttct

SEQ ID NO: 9 - DNA, 21 bp, Artificial Sequence
  Forward primer for mouse CD80
tcaatacgactcgcaaccaca

SEQ ID NO: 10 - DNA, 20 bp, Artificial Sequence
  Reverse primer for mouse CD80
gagggtcttctgggggtttt

SEQ ID NO: 11 - DNA, 20 bp, Artificial Sequence
  Forward primer for mouse 4-1BBL
acctgggtacccgagagaat

SEQ ID NO: 12 - DNA, 20 bp, Artificial Sequence
  Reverse primer for mouse 4-1BBL
gtagcttggcgaacacagga

SEQ ID NO: 13 - DNA, 20 bp, Artificial Sequence
  Forward primer for mouse OX40L
agaagacgctaaggctggtg

SEQ ID NO: 14 - DNA, 20 bp, Artificial Sequence
  Reverse primer for mouse OX40L
gccggagaggaagagagttg

SEQ ID NO: 15 - DNA, 20 bp, Artificial Sequence
  Forward primer for mouse CD70
ccgcacacagctgagttaca

SEQ ID NO: 16 - DNA, 20 bp, Artificial Sequence
  Reverse primer for mouse CD70
ctctggtccgtgtgtgaagg

SEQ ID NO: 17 - DNA, 20 bp, Artificial Sequence
  Forward primer for mouse CD86
aaagaggagcaagcagacgc

SEQ ID NO: 18 - DNA, 21 bp, Artificial Sequence
  Reverse primer for mouse CD86
catggtgcatctggggtccat

SEQ ID NO: 19 - DNA, 20 bp, Artificial Sequence
  Forward primer for mouse IRF1
gaaagtccaagtccagccga

SEQ ID NO: 20 - DNA, 20 bp, Artificial Sequence
  Reverse primer for mouse IRF1
gctgtggtcatcaggtaggg

SEQ ID NO: 21 - DNA, 20 bp, Artificial Sequence
  Forward primer for mouse IL-2
gaaactccccaggatgctca

SEQ ID NO: 22 - DNA, 21 bp, Artificial Sequence
  Reverse primer for mouse IL-2
cgcagaggtccaagttcatct

SEQ ID NO: 23 - DNA, 20 bp, Artificial Sequence
  Forward primer for mouse GAPDH
ccactcacggcaaattcaac

SEQ ID NO: 24 - DNA, 20 bp, Artificial Sequence
  Reverse primer for mouse GAPDH
ctccacgacatactcagcac

SEQ ID NO: 25 - RNA, 58 nt, Artificial Sequence
  DRG2-shRNA
ccgggctcatcctacatgaatacaactcgagttgtattcatgtaggatgagctttttg

SEQ ID NO: 26 - RNA, 23 nt, Artificial Sequence
  siDRG2
cauugaauacaaaggugccaaca